European Patent Specification EP 4 188 545 B1, published January 31, 2024. Title: Composition for treating damaged epithelial surfaces and method of producing same. Applicant: SerEye GmbH. The sequence listing filed with the application follows.

SEQUENCE LISTING (6 sequences)

SEQ ID NO: 1 - DNA, 23 bp, Artificial Sequence
  Primer MMP-9 forward
agtaccgaagagaaagcctactt

SEQ ID NO: 2 - DNA, 20 bp, Artificial Sequence
  Primer MMP-9 reverse
tgcaggatgtcaaagctcac

SEQ ID NO: 3 - DNA, 18 bp, Artificial Sequence
  Primer GAPDH forward
gaaggtgaaggtcggagt

SEQ ID NO: 4 - DNA, 20 bp, Artificial Sequence
  Primer GAPDH reverse
gaagatggtgatgggatttc

SEQ ID NO: 5 - DNA, 19 bp, Artificial Sequence
  Primer beta-actin forward
gctatttggcdctggactt

SEQ ID NO: 6 - DNA, 19 bp, Artificial Sequence
  Primer beta-actin reverse
gcggctcgtagctcttctc